European Patent Application EP 4 410 812 A1, published August 7, 2024. Title: Peptide having hair loss preventing activity or hair growth promoting activity and use thereof. Applicant: CAREGENE CO., LTD. The sequence listing filed with the application follows.

SEQUENCE LISTING (17 sequences)

SEQ ID NO: 1 - protein, 5 aa, synthetic construct
GGVPG

SEQ ID NO: 2 - DNA, 20 bp, synthetic construct
  source 1..20: mol_type = other DNA
ccagctattgtaacacctca

SEQ ID NO: 3 - DNA, 20 bp, synthetic construct
  source 1..20: mol_type = other DNA
ttcagatgtaggcagctgtc

SEQ ID NO: 4 - DNA, 25 bp, synthetic construct
  source 1..25: mol_type = other DNA
accagcagcgactctgaggaggaac

SEQ ID NO: 5 - DNA, 26 bp, synthetic construct
  source 1..26: mol_type = other DNA
tgaccctcttggcagcaggatagtcc

SEQ ID NO: 6 - DNA, 28 bp, synthetic construct
  source 1..28: mol_type = other DNA
accttcgttgccctctgtgccacagatg

SEQ ID NO: 7 - DNA, 21 bp, synthetic construct
  source 1..21: mol_type = other DNA
aggcccggaggcagtccgggt

SEQ ID NO: 8 - DNA, 20 bp, synthetic construct
  source 1..20: mol_type = other DNA
ggagccaaaagggtcatcat

SEQ ID NO: 9 - DNA, 20 bp, synthetic construct
  source 1..20: mol_type = other DNA
gtgatggcatggactgtggt

SEQ ID NO: 10 - DNA, 20 bp, synthetic construct
  source 1..20: mol_type = other DNA
gatcatcgagctgagacgca

SEQ ID NO: 11 - DNA, 20 bp, synthetic construct
  source 1..20: mol_type = other DNA
ctggccccagggtatctagt

SEQ ID NO: 12 - DNA, 20 bp, synthetic construct
  source 1..20: mol_type = other DNA
ccaaatccgcaccaaggtca

SEQ ID NO: 13 - DNA, 21 bp, synthetic construct
  source 1..21: mol_type = other DNA
gtattgattgccaggaggggg

SEQ ID NO: 14 - DNA, 20 bp, synthetic construct
  source 1..20: mol_type = other DNA
cgcggcgtatccgtgtcctc

SEQ ID NO: 15 - DNA, 24 bp, synthetic construct
  source 1..24: mol_type = other DNA
agcctgttccgtctcaaacttggt

SEQ ID NO: 16 - DNA, 20 bp, synthetic construct
  source 1..20: mol_type = other DNA
cggtcaagtcggaaaattca

SEQ ID NO: 17 - DNA, 20 bp, synthetic construct
  source 1..20: mol_type = other DNA
gaggagctgggatgtggtaa